European Patent Application EP 4 616 866 A1, published September 17, 2025. Title: AGENT FOR PREVENTING OR TREATING DISEASE ASSOCIATED WITH ACCUMULATION OF ABNORMAL PROTEIN AGGREGATES. Applicant: Osaka University. Application WO PCT/JP2023/040020, filed November 7, 2023. The sequence listing filed with the application follows.

SEQUENCE LISTING (62 sequences)

SEQ ID NO: 1 - protein, 450 aa, Homo sapiens
MQPPRERLVVTGRAGWMGMGRGAGRSALGFWPTLAFLLCSFPAATSPCKILKCNSEFWSATSGSHAPASDDTPEFCAALRSYALCTRRTARTCRGDLAYHSAVHGIEDLMSQHNCSKDGPTSQPRLRTLPPAGDSQERSDSPEICHYEKSFHKHSATPNYTHCGLFGDPHLRTFTDRFQTCKVQGAWPLIDNNYLNVQVTNTPVLPGSAATATSKLTIIFKNFQECVDQKVYQAEMDELPAAFVDGSKNGGDKHGANSLKITEKVSGQHVEIQAKYIGTTIVVRQVGRYLTFAVRMPEEVVNAVEDWDSQGLYLCLRGCPLNQQIDFQAFHTNAEGTGARRLAAASPAPTAPETFPYETAVAKCKEKLPVEDLYYQACVFDLLTTGDVNFTLAAYYALEDVKMLHSNKDKLHLYERTRDLPGRAAAGLPLAPRPLLGALVPLLALLPVFC

SEQ ID NO: 2 - protein, 454 aa, Mus musculus
MQPPRERLVVTGRAGWMGMGRGAGRSALGLWPTLAFLLCSFPAAISPCKILKCNSEFWSATSSGSHAPASDDVPEFCAALRTYALCTRRTARTCRGDLAYHSAVHGIEDLMSQHNCSKDGPTSQPRVRTLPPAGDSQERSDSPEICHYEKSFHKHSAAPNYTHCGLFGDPHLRTFTDHFQTCKVQGAWPLIDNNYLNVQVTNTPVLPGSAATATSKLTIIFKNFQECVDQKVYQAEMDELPSAFADGSKNGGDKHGANSLKITEKVSGQHVEIQAKYIGTTIVVRQVGRYLTFAVRMPEEVVNAVEDRDSQGLYLCLRGCPLNQQIDFQAFRANAESPRRPAAASPSPVVPETFPYETAVAKCKEKLPVEDLYYQACVFDLLTTGDVNFTLAAYYALEDGKMLHSNKDKLHLFERTRELPGAVAAAAAAATTFPLAPQILLGTIPLLVLLPVLW

SEQ ID NO: 3 - protein, 449 aa, Rattus norvegicus
MQPPRERLVVTGRAGWMGMGRGAGRSALGLWPTLAFLLCSFPAAISPCKILKCNSEFWSATSSGSHAPASDDVPEFCAALRTYALCTRRTARTCRGDLAYHSAVHGIEDLMSQHNCSKDGPTSQPRVRTLPPAGDSQERSDSPEICHYEKSFHKHSAAPNYTHCGLFGDPHLRTFTDHFQTCKVQGAWPLIDNNYLNVQVTNTPVLPGSAATATSKLTIIFKNFQECVDQKVYQAEMDELPSAFADGSKNGGDKHGANSLKITEKVSGQHVEIQAKYIGTTIVVRQVGRYLTFAVRMPEEVVNAVEDRDSQGLYLCLRGCPLNQQIDFQAFRANAESPRRPAAASPSPVVPETFPYETAVAKCKEKLPVEDLYYQACVFDLLTTGDVNFTLAAYYALEDGKMLHSNKDKLHLFERTRELPGAVAAAAFPLAPEMLPGTVTLLVLLPLFW

SEQ ID NO: 4 - DNA, 1353 bp, Homo sapiens
  source 1..1353: mol_type = genomic DNA
atgcagccgccaagggagaggctagtggtaacaggccgagctggatggatgggtatggggagaggggcaggacgttcagccctgggattctggccgaccctcgccttccttctctgcagcttccccgcagccacctccccgtgcaagatcctcaagtgcaactctgagttctggagcgccacgtcgggcagccacgccccagcctcagacgacacccccgagttctgtgcagccttgcgcagctacgccctgtgcacgcggcggacggcccgcacctgccggggtgacctggcctaccactcggccgtccatggcatagaggacctcatgagccagcacaactgctccaaggatggccccacctcgcagccacgcctgcgcacgctcccaccggccggagacagccaggagcgctcggacagccccgagatctgccattacgagaagagctttcacaagcactcggccacccccaactacacgcactgtggcctcttcggggacccacacctcaggactttcaccgaccgcttccagacctgcaaggtgcagggcgcctggccgctcatcgacaataattacctgaacgtgcaggtcaccaacacgcctgtgctgcccggctcagcggccactgccaccagcaagctcaccatcatcttcaagaacttccaggagtgtgtggaccagaaggtgtaccaggctgagatggacgagctcccggccgccttcgtggatggctctaagaacggtggggacaagcacggggccaacagcctgaagatcactgagaaggtgtcaggccagcacgtggagatccaggccaagtacatcggcaccaccatcgtggtgcgccaggtgggccgctacctgacctttgccgtccgcatgccagaggaagtggtcaatgctgtggaggactgggacagccagggtctctacctctgcctgcggggctgccccctcaaccagcagatcgacttccaggccttccacaccaatgctgagggcaccggtgcccgcaggctggcagccgccagccctgcacccacagcccccgagaccttcccatacgagacagccgtggccaagtgcaaggagaagctgccggtggaggacctgtactaccaggcctgcgtcttcgacctcctcaccacgggcgacgtgaacttcacactggccgcctactacgcgttggaggatgtcaagatgctccactccaacaaagacaaactgcacctgtatgagaggactcgggacctgccaggcagggcggctgcggggctgcccctggccccccggcccctcctgggcgccctcgtcccgctcctggccctgctccctgtgttctgctag

SEQ ID NO: 5 - protein, 6 aa, Mus musculus
QDISSY

SEQ ID NO: 6 - skipped

SEQ ID NO: 7 - protein, 9 aa, Mus musculus
QQLNTLPWT

SEQ ID NO: 8 - protein, 8 aa, Mus musculus
GFTFSDAW

SEQ ID NO: 9 - protein, 10 aa, Mus musculus
IRSKANNHAT

SEQ ID NO: 10 - protein, 7 aa, Mus musculus
TRRDGAY

SEQ ID NO: 11 - protein, 11 aa, Mus musculus
QSLVHSNGNTY

SEQ ID NO: 12 - skipped

SEQ ID NO: 13 - protein, 9 aa, Mus musculus
SQSTHVPYT

SEQ ID NO: 14 - protein, 9 aa, Mus musculus
GYSITTSYY

SEQ ID NO: 15 - protein, 7 aa, Mus musculus
ISYDGTN

SEQ ID NO: 16 - protein, 23 aa, Homo sapiens
PCKILKCNSEFWSATSGSHAPAS

SEQ ID NO: 17 - protein, 16 aa, synthetic construct
  REGION 1..16: note = Description of Artificial Sequence: Syntheticpeptide
RSSQSLEYSDGYTFLE

SEQ ID NO: 18 - protein, 7 aa, synthetic construct
  REGION 1..7: note = Description of Artificial Sequence: Syntheticpeptide
EVSNRFS

SEQ ID NO: 19 - protein, 9 aa, synthetic construct
  REGION 1..9: note = Description of Artificial Sequence: Syntheticpeptide
FQATHDPLT

SEQ ID NO: 20 - protein, 5 aa, synthetic construct
  REGION 1..5: note = Description of Artificial Sequence: Syntheticpeptide
NYGMN

SEQ ID NO: 21 - protein, 17 aa, synthetic construct
  REGION 1..17: note = Description of Artificial Sequence: Syntheticpeptide
MIYYDSSEKHYADSVKG

SEQ ID NO: 22 - protein, 6 aa, synthetic construct
  REGION 1..6: note = Description of Artificial Sequence: Syntheticpeptide
GTTPDY

SEQ ID NO: 23 - protein, 11 aa, synthetic construct
  REGION 1..11: note = Description of Artificial Sequence: Syntheticpeptide
QASQDIDNYLA

SEQ ID NO: 24 - protein, 7 aa, synthetic construct
  REGION 1..7: note = Description of Artificial Sequence: Syntheticpeptide
GATNLAD

SEQ ID NO: 25 - protein, 9 aa, synthetic construct
  REGION 1..9: note = Description of Artificial Sequence: Syntheticpeptide
LQGYIPPRT

SEQ ID NO: 26 - protein, 5 aa, synthetic construct
  REGION 1..5: note = Description of Artificial Sequence: Syntheticpeptide
SYVMH

SEQ ID NO: 27 - protein, 17 aa, synthetic construct
  REGION 1..17: note = Description of Artificial Sequence: Syntheticpeptide
YIIPYNDNTKYNEKFKG

SEQ ID NO: 28 - protein, 14 aa, synthetic construct
  REGION 1..14: note = Description of Artificial Sequence: Syntheticpeptide
ARRNEYYGSSFFDY

SEQ ID NO: 29 - protein, 14 aa, synthetic construct
  REGION 1..14: note = Description of Artificial Sequence: Syntheticpeptide
TGTSSSVGDSIYVS

SEQ ID NO: 30 - protein, 7 aa, synthetic construct
  REGION 1..7: note = Description of Artificial Sequence: Syntheticpeptide
DVTKRPS

SEQ ID NO: 31 - protein, 9 aa, synthetic construct
  REGION 1..9: note = Description of Artificial Sequence: Syntheticpeptide
CSYAGTDTL

SEQ ID NO: 32 - protein, 5 aa, synthetic construct
  REGION 1..5: note = Description of Artificial Sequence: Syntheticpeptide
SHGIS

SEQ ID NO: 33 - protein, 17 aa, synthetic construct
  REGION 1..17: note = Description of Artificial Sequence: Syntheticpeptide
WISPYSGNTNYAQKLQG

SEQ ID NO: 34 - protein, 11 aa, synthetic construct
  REGION 1..11: note = Description of Artificial Sequence: Syntheticpeptide
VGSGPYYYMDV

SEQ ID NO: 35 - protein, 9 aa, synthetic construct
  REGION 1..9: note = Description of Artificial Sequence: Syntheticpeptide
YSYAGTDTL

SEQ ID NO: 36 - protein, 14 aa, Homo sapiens
EEVVNAVEDWDSQG

SEQ ID NO: 37 - protein, 14 aa, Homo sapiens
NQQIDFQAFHTNAE

SEQ ID NO: 38 - protein, 11 aa, Homo sapiens
PTAPETFPYET

SEQ ID NO: 39 - protein, 11 aa, Homo sapiens
KLPVEDLYYQA

SEQ ID NO: 40 - protein, 9 aa, synthetic construct
  REGION 1..9: note = Description of Artificial Sequence: Syntheticpeptide
FSYAGTDTL

SEQ ID NO: 41 - protein, 9 aa, synthetic construct
  REGION 1..9: note = Description of Artificial Sequence: Syntheticpeptide
HSYAGTDTL

SEQ ID NO: 42 - protein, 9 aa, synthetic construct
  REGION 1..9: note = Description of Artificial Sequence: Syntheticpeptide
LSYAGTDTL

SEQ ID NO: 43 - protein, 9 aa, synthetic construct
  REGION 1..9: note = Description of Artificial Sequence: Syntheticpeptide
VSYAGTDTL

SEQ ID NO: 44 - protein, 9 aa, synthetic construct
  REGION 1..9: note = Description of Artificial Sequence: Syntheticpeptide
ISYAGTDTL

SEQ ID NO: 45 - protein, 9 aa, synthetic construct
  REGION 1..9: note = Description of Artificial Sequence: Syntheticpeptide
KSYAGTDTL

SEQ ID NO: 46 - protein, 107 aa, synthetic construct
  REGION 1..107: note = humanized antibody light chain
DIQMTQSPSSVSASVGDRVTITCRASQDISSYLNWYQQKPGKAPKLLIYYTSRLHSGVPSRFSGSGSGTDFTLTISSLQPEDFASYFCQQLNTLPWTFGGGTKVEME

SEQ ID NO: 47 - protein, 116 aa, synthetic construct
  REGION 1..116: note = humanized antibody heavy chain
EVQLVESGGGLVQPGRSLRLSCTASGFTFSDAWMDWVRQAPGKGLEWVAEIRSKANNHATYYAESVKGRFTISRDDSKSIVYLQMNSLRTEDTALYYCTRRDGAYWGKGTTVTVSS

SEQ ID NO: 48 - protein, 214 aa, synthetic construct
  REGION 1..214: note = humanized antibody light chain KA
DIQMTQSPSSVSASVGDRVTITCRASQDISSYLNWYQQKPGKAPKLLIYYTSRLHSGVPSRFSGSGSGTDFTLTISSLQPEDFASYFCQQLNTLPWTFGGGTKVEMERTVAAPSVFIFPPSDEQLKSGTASVVCLLNNFYPREAKVQWKVDNALQSGNSQESVTEQDSKDSTYSLSSTLTLSKADYEKHKVYACEVTHQGLSSPVTKSFNRGEC

SEQ ID NO: 49 - protein, 446 aa, synthetic construct
  REGION 1..446: note = humanized antibody heavy chain HE
EVQLVESGGGLVQPGRSLRLSCTASGFTFSDAWMDWVRQAPGKGLEWVAEIRSKANNHATYYAESVKGRFTISRDDSKSIVYLQMNSLRTEDTALYYCTRRDGAYWGKGTTVTVSSASTKGPSVFPLAPSSKSTSGGTAALGCLVKDYFPEPVTVSWNSGALTSGVHTFPAVLQSSGLYSLSSVVTVPSSSLGTQTYICNVNHKPSNTKVDKKVEPKSCDKTHTCPPCPAPELLGGPSVFLFPPKPKDTLMISRTPEVTCVVVDVSHEDPEVKFNWYVDGVEVHNAKTKPREEQYNSTYRVVSVLTVLHQDWLNGKEYKCKVSNKALPAPIEKTISKAKGQPREPQVYTLPPSRDELTKNQVSLTCLVKGFYPSDIAVEWESNGQPENNYKTTPPVLDSDGSFFLYSKLTVDKSRWQQGNVFSCSVMHEALHNHYTQKSLSLSPGK

SEQ ID NO: 50 - protein, 112 aa, Mus musculus
DVVMTQTPLSLPVSLGDQASISCRSSQSLVHSNGNTYLHWYLQRPGQSPKLLIYKVSNRFSGVPDRFSGSGSGTDFTLKISRVEAEDLGLYFCSQSTHVPYTFGGGTKLEIK

SEQ ID NO: 51 - protein, 112 aa, Mus musculus
DVKLQESGPGLVKPSQSLSLTCSVTGYSITTSYYWNWIRQFPGNKLEWMGYISYDGTNNYNPSLKNRISITRDTSKNQFFLRLNSVTTEDTATYYCAGSFGYSQGTLVTVSA

SEQ ID NO: 52 - protein, 238 aa, Mus musculus
MKLPVRLLVLMFWIPASSSDVVMTQTPLSLPVSLGDQASISCRSSQSLVHSNGNTYLHWYLQRPGQSPKLLIYKVSNRFSGVPDRFSGSGSGTDFTLKISRVEAEDLGLYFCSQSTHVPYTFGGGTKLEIKRADAAPTVSIFPPSSEQLTSGGASVVCFLNNFYPKDINVKWKIDGSERQNGVLNSWTDQDSKDSTYSMSSTLTLTKDEYERHNSYTCEATHKTSTSPIVKSFNRNEC

SEQ ID NO: 53 - protein, 466 aa, Mus musculus
MKVLSLLYLLTAIPGIMSDVKLQESGPGLVKPSQSLSLTCSVTGYSITTSYYWNWIRQFPGNKLEWMGYISYDGTNNYNPSLKNRISITRDTSKNQFFLRLNSVTTEDTATYYCAGSFGYSQGTLVTVSAAKTTPPSVYPLAPGCGDTTGSSVTLGCLVKGYFPESVTVTWNSGSLSSSVHTFPALLQSGLYTMSSSVTVPSSTWPSQTVTCSVAHPASSTTVDKKLEPSGPISTINPCPPCKECHKCPAPNLEGGPSVFIFPPNIKDVLMISLTPKVTCVVVDVSEDDPDVQISWFVNNVEVHTAQTQTHREDYNSTIRVVSTLPIQHQDWMSGKEFKCKVNNKDLPSPIERTISKIKGLVRAPQVYILPPPAEQLSRKDVSLTCLVVGFNPGDISVEWTSNGHTEENYKDTAPVLDSDGSYFIYSKLNMKTSKWEKTDSFSCNVRHEGLKNYYLKKTISRSPGK

SEQ ID NO: 54 - protein, 113 aa, synthetic construct
  REGION 1..113: note = VL 5F9
DVVLTQTPVSLSVTLGDQASMSCRSSQSLEYSDGYTFLEWFLQKPGQSPQLLIYEVSNRFSGVPDRFIGSGSGTDFTLKISRVEPEDLGVYYCFQATHDPLTFGSGTKLEIKR

SEQ ID NO: 55 - protein, 115 aa, synthetic construct
  REGION 1..115: note = VH 5F9
EVQLVESGGGLVQPGSSLKLSCVASGFTFSNYGMNWIRQAPKKGLEWIGMIYYDSSEKHYADSVKGRFTISRDNSKNTLYLEMNSLRSEDTAIYYCAKGTTPDYWGQGVMVTVSS

SEQ ID NO: 56 - protein, 108 aa, synthetic construct
  REGION 1..108: note = VL 8D1
DIQMTQSPASLSASLEEIVTITCQASQDIDNYLAWYHQKPGKSPRLLIYGATNLADGVPSRFSGSRSGTQFSLKINRLQIEDLGIYYCLQGYIPPRTFGGGTKLELKR

SEQ ID NO: 57 - protein, 121 aa, synthetic construct
  REGION 1..121: note = VH 8D1
EVQLQQSGPELVKPGTSVKMSCKTSGYTFTSYVMHWVKQKPGQGLEWIGYIIPYNDNTKYNEKFKGKATLTSDKSSSTAYMELSSLTSEDSAVYYCARRNEYYGSSFFDYWGQGTTLTVSS

SEQ ID NO: 58 - protein, 109 aa, synthetic construct
  REGION 1..109: note = Description of Artificial Sequence: Syntheticpolypeptide
QSALTQPRSVSGSPGQSVTISCTGTSSSVGDSIYVSWYQQHPGKAPKLMLYDVTKRPSGVPDRFSGSKSGNTASLTISGLQAEDEADYYCCSYAGTDTLFGGGTKVTVL

SEQ ID NO: 59 - protein, 120 aa, synthetic construct
  REGION 1..120: note = Description of Artificial Sequence: Syntheticpolypeptide
EVQLVQSGAEVKKPGASVKVSCKASGYTFTSHGISWVRQAPGQGLDWMGWISPYSGNTNYAQKLQGRVTMTTDTSTSTAYMELSSLRSEDTAVYYCARVGSGPYYYMDVWGQGTLVTVSS

SEQ ID NO: 60 - protein, 109 aa, synthetic construct; identical to SEQ ID NO: 58
  REGION 1..109: note = Description of Artificial Sequence: Syntheticpolypeptide

SEQ ID NO: 61 - protein, 215 aa, synthetic construct
  REGION 1..215: note = Description of Artificial Sequence: Syntheticpolypeptide
QSALTQPRSVSGSPGQSVTISCTGTSSSVGDSIYVSWYQQHPGKAPKLMLYDVTKRPSGVPDRFSGSKSGNTASLTISGLQAEDEADYYCYSYAGTDTLFGGGTKVTVLGQPKAAPSVTLFPPSSEELQANKATLVCLISDFYPGAVTVAWKADSSPVKAGVETTTPSKQSNNKYAASSYLSLTPEQWKSHRSYSCQVTHEGSTVEKTVAPTECS

SEQ ID NO: 62 - protein, 450 aa, synthetic construct
  REGION 1..450: note = Description of Artificial Sequence: Syntheticpolypeptide
EVQLVQSGAEVKKPGASVKVSCKASGYTFTSHGISWVRQAPGQGLDWMGWISPYSGNTNYAQKLQGRVTMTTDTSTSTAYMELSSLRSEDTAVYYCARVGSGPYYYMDVWGQGTLVTVSSASTKGPSVFPLAPSSKSTSGGTAALGCLVKDYFPEPVTVSWNSGALTSGVHTFPAVLQSSGLYSLSSVVTVPSSSLGTQTYICNVNHKPSNTKVDKKVEPKSCDKTHTCPPCPAPEAAGGPSVFLFPPKPKDQLMISRTPEVTCVVVDVSHEDPEVKFNWYVDGVEVHNAKTKPREEQYNSTYRVVSVLTVLHQDWLNGKEYKCKVSNKALPAPIEKTISKAKGQPREPQVYTLPPSREEMTKNQVSLTCLVKGFYPSDIAVEWESNGQPENNYKTTPPVLDSDGSFFLYSKLTVDKSRWQQGNVFSCSVLHEALHNHYTQKSLSLSPGK